European Patent Specification EP 3 269 725 B1, published May 13, 2026. Title: METHOD FOR PRODUCING PROTEIN COMPOSITION, AND PROTEIN COMPOSITION. Applicant: SANYO CHEMICAL INDUSTRIES, LTD. The sequence listing filed with the application follows.

SEQUENCE LISTING (35 sequences)

SEQ ID NO: 1 - protein, 6 aa, Bombyx mori
GAGAGS

SEQ ID NO: 2 - protein, 5 aa, Homo sapiens
YIGSR

SEQ ID NO: 3 - protein, 5 aa, Homo sapiens
GVGVP

SEQ ID NO: 4 - protein, 5 aa, Homo sapiens
PGVGV

SEQ ID NO: 5 - protein, 5 aa, Homo sapiens
VPGVG

SEQ ID NO: 6 - protein, 5 aa, Homo sapiens
GVPGV

SEQ ID NO: 7 - protein, 5 aa, Homo sapiens
VGVPG

SEQ ID NO: 8 - protein, 9 aa, Homo sapiens
GAHGPAGPK

SEQ ID NO: 9 - protein, 5 aa, Bombyx mori
VAAGY

SEQ ID NO: 10 - protein, 7 aa, Bombyx mori
GAGAGAS

SEQ ID NO: 11 - protein, 6 aa, Homo sapiens
LGPLGP

SEQ ID NO: 12 - protein, 9 aa, Homo sapiens
GAHGPAGPK

SEQ ID NO: 13 - protein, 18 aa, Homo sapiens
GAPGPAGPPGSRGDPGPP

SEQ ID NO: 14 - protein, 9 aa, Homo sapiens
GAQGPAGPG

SEQ ID NO: 15 - protein, 15 aa, Homo sapiens
GAPGAPGSQGAPGLQ

SEQ ID NO: 16 - protein, 15 aa, Homo sapiens
GAPGTPGPQGLPGSP

SEQ ID NO: 17 - protein, 17 aa, Homo sapiens
GAAVTGRGDSPASAAGY

SEQ ID NO: 18 - protein, 20 aa, Homo sapiens
GAAPGASIKVAVSAGPSAGY

SEQ ID NO: 19 - protein, 24 aa, Artificial Sequence
  Repeat sequence
GAGAGSGAGAGSGAGAGSGAGAGS

SEQ ID NO: 20 - protein, 40 aa, Artificial Sequence
  Repeat sequence
GVGVPGVGVPGVGVPGVGVPGKGVPGVGVPGVGVPGVGVP

SEQ ID NO: 21 - protein, 12 aa, Artificial Sequence
  Repeat sequence
GAGAGSGAGAGS

SEQ ID NO: 22 - protein, 874 aa, Artificial Sequence
  SELP8K
MDPVVLQRRDWENPGVTQLNRLAAHPPFASDPMGVGVPGVGVPGVGVPGVGVPGKGVPGVGVPGVGVPGVGVPGAGAGSGAGAGSGAGAGSGAGAGSGVGVPGVGVPGVGVPGVGVPGKGVPGVGVPGVGVPGVGVPGAGAGSGAGAGSGAGAGSGAGAGSGVGVPGVGVPGVGVPGVGVPGKGVPGVGVPGVGVPGVGVPGAGAGSGAGAGSGAGAGSGAGAGSGVGVPGVGVPGVGVPGVGVPGKGVPGVGVPGVGVPGVGVPGAGAGSGAGAGSGAGAGSGAGAGSGVGVPGVGVPGVGVPGVGVPGKGVPGVGVPGVGVPGVGVPGAGAGSGAGAGSGAGAGSGAGAGSGVGVPGVGVPGVGVPGVGVPGKGVPGVGVPGVGVPGVGVPGAGAGSGAGAGSGAGAGSGAGAGSGVGVPGVGVPGVGVPGVGVPGKGVPGVGVPGVGVPGVGVPGAGAGSGAGAGSGAGAGSGAGAGSGVGVPGVGVPGVGVPGVGVPGKGVPGVGVPGVGVPGVGVPGAGAGSGAGAGSGAGAGSGAGAGSGVGVPGVGVPGVGVPGVGVPGKGVPGVGVPGVGVPGVGVPGAGAGSGAGAGSGAGAGSGAGAGSGVGVPGVGVPGVGVPGVGVPGKGVPGVGVPGVGVPGVGVPGAGAGSGAGAGSGAGAGSGAGAGSGVGVPGVGVPGVGVPGVGVPGKGVPGVGVPGVGVPGVGVPGAGAGSGAGAGSGAGAGSGAGAGSGVGVPGVGVPGVGVPGVGVPGKGVPGVGVPGVGVPGVGVPGAGAGSGAGAGSGAGAGSGAGAGSGVGVPGVGVPGVGVPGVGVPGKGVPGVGVPGVGVPGVGVPGAGAGSGAGAGSGAGAMDPGRYQDLRSHHHHHH

SEQ ID NO: 23 - protein, 938 aa, Artificial Sequence
  SELP0K
MDPVVLQRRDWENPGVTQLNRLAAHPPFASDPMGVGVPGVGVPGVGVPGVGVPGKGVPGVGVPGVGVPGVGVPGAGAGSGAGAGSGVGVPGVGVPGVGVPGVGVPGKGVPGVGVPGVGVPGVGVPGAGAGSGAGAGSGVGVPGVGVPGVGVPGVGVPGKGVPGVGVPGVGVPGVGVPGAGAGSGAGAGSGVGVPGVGVPGVGVPGVGVPGKGVPGVGVPGVGVPGVGVPGAGAGSGAGAGSGVGVPGVGVPGVGVPGVGVPGKGVPGVGVPGVGVPGVGVPGAGAGSGAGAGSGVGVPGVGVPGVGVPGVGVPGKGVPGVGVPGVGVPGVGVPGAGAGSGAGAGSGVGVPGVGVPGVGVPGVGVPGKGVPGVGVPGVGVPGVGVPGAGAGSGAGAGSGVGVPGVGVPGVGVPGVGVPGKGVPGVGVPGVGVPGVGVPGAGAGSGAGAGSGVGVPGVGVPGVGVPGVGVPGKGVPGVGVPGVGVPGVGVPGAGAGSGAGAGSGVGVPGVGVPGVGVPGVGVPGKGVPGVGVPGVGVPGVGVPGAGAGSGAGAGSGVGVPGVGVPGVGVPGVGVPGKGVPGVGVPGVGVPGVGVPGAGAGSGAGAGSGVGVPGVGVPGVGVPGVGVPGKGVPGVGVPGVGVPGVGVPGAGAGSGAGAGSGVGVPGVGVPGVGVPGVGVPGKGVPGVGVPGVGVPGVGVPGAGAGSGAGAGSGVGVPGVGVPGVGVPGVGVPGKGVPGVGVPGVGVPGVGVPGAGAGSGAGAGSGVGVPGVGVPGVGVPGVGVPGKGVPGVGVPGVGVPGVGVPGAGAGSGAGAGSGVGVPGVGVPGVGVPGVGVPGKGVPGVGVPGVGVPGVGVPGAGAGSGAGAGSGVGVPGVGVPGVGVPGVGVPGKGVPGVGVPGVGVPGVGVPGAGAGSGAGAGSGAGAMDPGRYQDLRSHHHHHH

SEQ ID NO: 24 - protein, 60 aa, Artificial Sequence
  Repeat sequence
GVGVPGVGVPGVGVPGVGVPGKGVPGVGVPGVGVPGVGVPGVGVPGVGVPGVGVPGVGVP

SEQ ID NO: 25 - protein, 886 aa, Artificial Sequence
  SELP415K
MDPVVLQRRDWENPGVTQLNRLAAHPPFASDPMGAGAGSGAGAGSGVGVPGVGVPGVGVPGVGVPGKGVPGVGVPGVGVPGVGVPGVGVPGVGVPGVGVPGVGVPGVGVPGVGVPGVGVPGVGVPGAGAGSGAGAGSGAGAGSGAGAGSGVGVPGVGVPGVGVPGVGVPGKGVPGVGVPGVGVPGVGVPGVGVPGVGVPGVGVPGVGVPGVGVPGVGVPGVGVPGVGVPGAGAGSGAGAGSGAGAGSGAGAGSGVGVPGVGVPGVGVPGVGVPGKGVPGVGVPGVGVPGVGVPGVGVPGVGVPGVGVPGVGVPGVGVPGVGVPGVGVPGVGVPGAGAGSGAGAGSGAGAGSGAGAGSGVGVPGVGVPGVGVPGVGVPGKGVPGVGVPGVGVPGVGVPGVGVPGVGVPGVGVPGVGVPGVGVPGVGVPGVGVPGVGVPGAGAGSGAGAGSGAGAGSGAGAGSGVGVPGVGVPGVGVPGVGVPGKGVPGVGVPGVGVPGVGVPGVGVPGVGVPGVGVPGVGVPGVGVPGVGVPGVGVPGVGVPGAGAGSGAGAGSGAGAGSGAGAGSGVGVPGVGVPGVGVPGVGVPGKGVPGVGVPGVGVPGVGVPGVGVPGVGVPGVGVPGVGVPGVGVPGVGVPGVGVPGVGVPGAGAGSGAGAGSGAGAGSGAGAGSGVGVPGVGVPGVGVPGVGVPGKGVPGVGVPGVGVPGVGVPGVGVPGVGVPGVGVPGVGVPGVGVPGVGVPGVGVPGVGVPGAGAGSGAGAGSGAGAGSGAGAGSGVGVPGVGVPGVGVPGVGVPGKGVPGVGVPGVGVPGVGVPGVGVPGVGVPGVGVPGVGVPGVGVPGVGVPGVGVPGVGVPGAGAGSGAGAGSGAGAMDPGRYQDLRSHHHHHH

SEQ ID NO: 26 - protein, 750 aa, Artificial Sequence
  SELP815K
MDPVVLQRRDWENPGVTQLNRLAAHPPFASDPMGAGAGSGAGAGSGVGVPGVGVPGVGVPGVGVPGKGVPGVGVPGVGVPGVGVPGVGVPGVGVPGVGVPGVGVPGVGVPGVGVPGVGVPGVGVPGAGAGSGAGAGSGAGAGSGAGAGSGAGAGSGAGAGSGVGVPGVGVPGVGVPGVGVPGKGVPGVGVPGVGVPGVGVPGVGVPGVGVPGVGVPGVGVPGVGVPGVGVPGVGVPGVGVPGAGAGSGAGAGSGAGAGSGAGAGSGAGAGSGAGAGSGVGVPGVGVPGVGVPGVGVPGKGVPGVGVPGVGVPGVGVPGVGVPGVGVPGVGVPGVGVPGVGVPGVGVPGVGVPGVGVPGAGAGSGAGAGSGAGAGSGAGAGSGAGAGSGAGAGSGVGVPGVGVPGVGVPGVGVPGKGVPGVGVPGVGVPGVGVPGVGVPGVGVPGVGVPGVGVPGVGVPGVGVPGVGVPGVGVPGAGAGSGAGAGSGAGAGSGAGAGSGAGAGSGAGAGSGVGVPGVGVPGVGVPGVGVPGKGVPGVGVPGVGVPGVGVPGVGVPGVGVPGVGVPGVGVPGVGVPGVGVPGVGVPGVGVPGAGAGSGAGAGSGAGAGSGAGAGSGAGAGSGAGAGSGVGVPGVGVPGVGVPGVGVPGKGVPGVGVPGVGVPGVGVPGVGVPGVGVPGVGVPGVGVPGVGVPGVGVPGVGVPGVGVPGAGAGSGAGAGSGAGAGSGAGAGSGAGAMDPGRYQDLRSHHHHHH

SEQ ID NO: 27 - protein, 36 aa, Artificial Sequence
  Repeat sequence
GAGAGSGAGAGSGAGAGSGAGAGSGAGAGSGAGAGS

SEQ ID NO: 28 - protein, 54 aa, Artificial Sequence
  Repeat sequence
GAGAGSGAGAGSGAGAGSGAGAGSGAGAGSGAGAGSGAGAGSGAGAGSGAGAGS

SEQ ID NO: 29 - protein, 852 aa, Artificial Sequence
  Repeat sequence
GAGAGSGAGAGSGAGAGSGAGAGSGAGAGSGAGAGSGAGAGSGAGAGSGAGAGSGAAVTGRGDSPASAAGYGAGAGSGAGAGSGAGAGSGAGAGSGAGAGSGAGAGSGAGAGSGAGAGSGAGAGSGAAVTGRGDSPASAAGYGAGAGSGAGAGSGAGAGSGAGAGSGAGAGSGAGAGSGAGAGSGAGAGSGAGAGSGAAVTGRGDSPASAAGYGAGAGSGAGAGSGAGAGSGAGAGSGAGAGSGAGAGSGAGAGSGAGAGSGAGAGSGAAVTGRGDSPASAAGYGAGAGSGAGAGSGAGAGSGAGAGSGAGAGSGAGAGSGAGAGSGAGAGSGAGAGSGAAVTGRGDSPASAAGYGAGAGSGAGAGSGAGAGSGAGAGSGAGAGSGAGAGSGAGAGSGAGAGSGAGAGSGAAVTGRGDSPASAAGYGAGAGSGAGAGSGAGAGSGAGAGSGAGAGSGAGAGSGAGAGSGAGAGSGAGAGSGAAVTGRGDSPASAAGYGAGAGSGAGAGSGAGAGSGAGAGSGAGAGSGAGAGSGAGAGSGAGAGSGAGAGSGAAVTGRGDSPASAAGYGAGAGSGAGAGSGAGAGSGAGAGSGAGAGSGAGAGSGAGAGSGAGAGSGAGAGSGAAVTGRGDSPASAAGYGAGAGSGAGAGSGAGAGSGAGAGSGAGAGSGAGAGSGAGAGSGAGAGSGAGAGSGAAVTGRGDSPASAAGYGAGAGSGAGAGSGAGAGSGAGAGSGAGAGSGAGAGSGAGAGSGAGAGSGAGAGSGAAVTGRGDSPASAAGYGAGAGSGAGAGSGAGAGSGAGAGSGAGAGSGAGAGSGAGAGSGAGAGSGAGAGSGAAVTGRGDSPASAAGY

SEQ ID NO: 30 - protein, 980 aa, Artificial Sequence
  PronectinF
MDPVVLQRRDWENPGVTQLNRLAAHPPFASDPMGAGSGAGAGSGAGAGSGAGAGSGAGAGSGAGAGSGAGAGSGAAVTGRGDSPASAAGYGAGAGSGAGAGSGAGAGSGAGAGSGAGAGSGAGAGSGAGAGSGAGAGSGAGAGSGAAVTGRGDSPASAAGYGAGAGSGAGAGSGAGAGSGAGAGSGAGAGSGAGAGSGAGAGSGAGAGSGAGAGSGAAVTGRGDSPASAAGYGAGAGSGAGAGSGAGAGSGAGAGSGAGAGSGAGAGSGAGAGSGAGAGSGAGAGSGAAVTGRGDSPASAAGYGAGAGSGAGAGSGAGAGSGAGAGSGAGAGSGAGAGSGAGAGSGAGAGSGAGAGSGAAVTGRGDSPASAAGYGAGAGSGAGAGSGAGAGSGAGAGSGAGAGSGAGAGSGAGAGSGAGAGSGAGAGSGAAVTGRGDSPASAAGYGAGAGSGAGAGSGAGAGSGAGAGSGAGAGSGAGAGSGAGAGSGAGAGSGAGAGSGAAVTGRGDSPASAAGYGAGAGSGAGAGSGAGAGSGAGAGSGAGAGSGAGAGSGAGAGSGAGAGSGAGAGSGAAVTGRGDSPASAAGYGAGAGSGAGAGSGAGAGSGAGAGSGAGAGSGAGAGSGAGAGSGAGAGSGAGAGSGAAVTGRGDSPASAAGYGAGAGSGAGAGSGAGAGSGAGAGSGAGAGSGAGAGSGAGAGSGAGAGSGAGAGSGAAVTGRGDSPASAAGYGAGAGSGAGAGSGAGAGSGAGAGSGAGAGSGAGAGSGAGAGSGAGAGSGAGAGSGAAVTGRGDSPASAAGYGAGAGSGAGAGSGAGAGSGAGAGSGAGAGSGAGAGSGAGAGSGAGAGSGAGAGSGAAVTGRGDSPASAAGYGAGAGSGAGAGSGAGAGSGAGAGSGAGAGSGAGAGSGAGAGSGAGAGSGAGAGSGAAVTGRGDSPASAAGYGAGAGSGAGAGSGAGAMDPGRYQLSAGRYHYQLVWCQK

SEQ ID NO: 31 - protein, 888 aa, Artificial Sequence
  Repeat sequence
GAGAGSGAGAGSGAGAGSGAGAGSGAGAGSGAGAGSGAGAGSGAGAGSGAGAGSGAAPGASIKVAVSAGPSAGYGAGAGSGAGAGSGAGAGSGAGAGSGAGAGSGAGAGSGAGAGSGAGAGSGAGAGSGAAPGASIKVAVSAGPSAGYGAGAGSGAGAGSGAGAGSGAGAGSGAGAGSGAGAGSGAGAGSGAGAGSGAGAGSGAAPGASIKVAVSAGPSAGYGAGAGSGAGAGSGAGAGSGAGAGSGAGAGSGAGAGSGAGAGSGAGAGSGAGAGSGAAPGASIKVAVSAGPSAGYGAGAGSGAGAGSGAGAGSGAGAGSGAGAGSGAGAGSGAGAGSGAGAGSGAGAGSGAAPGASIKVAVSAGPSAGYGAGAGSGAGAGSGAGAGSGAGAGSGAGAGSGAGAGSGAGAGSGAGAGSGAGAGSGAAPGASIKVAVSAGPSAGYGAGAGSGAGAGSGAGAGSGAGAGSGAGAGSGAGAGSGAGAGSGAGAGSGAGAGSGAAPGASIKVAVSAGPSAGYGAGAGSGAGAGSGAGAGSGAGAGSGAGAGSGAGAGSGAGAGSGAGAGSGAGAGSGAAPGASIKVAVSAGPSAGYGAGAGSGAGAGSGAGAGSGAGAGSGAGAGSGAGAGSGAGAGSGAGAGSGAGAGSGAAPGASIKVAVSAGPSAGYGAGAGSGAGAGSGAGAGSGAGAGSGAGAGSGAGAGSGAGAGSGAGAGSGAGAGSGAAPGASIKVAVSAGPSAGYGAGAGSGAGAGSGAGAGSGAGAGSGAGAGSGAGAGSGAGAGSGAGAGSGAGAGSGAAPGASIKVAVSAGPSAGYGAGAGSGAGAGSGAGAGSGAGAGSGAGAGSGAGAGSGAGAGSGAGAGSGAGAGSGAAPGASIKVAVSAGPSAGY

SEQ ID NO: 32 - protein, 1019 aa, Artificial Sequence
  PronectinL
MDPVVLQRRDWENPGVTQLNRLAAHPPFASDPMGAGSGAGAGSGAGAGSGAGAGSGAGAGSGAGAGSGAGAGSGAAPGASIKVAVSAGPSAGYGAGAGSGAGAGSGAGAGSGAGAGSGAGAGSGAGAGSGAGAGSGAGAGSGAGAGSGAAPGASIKVAVSAGPSAGYGAGAGSGAGAGSGAGAGSGAGAGSGAGAGSGAGAGSGAGAGSGAGAGSGAGAGSGAAPGASIKVAVSAGPSAGYGAGAGSGAGAGSGAGAGSGAGAGSGAGAGSGAGAGSGAGAGSGAGAGSGAGAGSGAAPGASIKVAVSAGPSAGYGAGAGSGAGAGSGAGAGSGAGAGSGAGAGSGAGAGSGAGAGSGAGAGSGAGAGSGAAPGASIKVAVSAGPSAGYGAGAGSGAGAGSGAGAGSGAGAGSGAGAGSGAGAGSGAGAGSGAGAGSGAGAGSGAAPGASIKVAVSAGPSAGYGAGAGSGAGAGSGAGAGSGAGAGSGAGAGSGAGAGSGAGAGSGAGAGSGAGAGSGAAPGASIKVAVSAGPSAGYGAGAGSGAGAGSGAGAGSGAGAGSGAGAGSGAGAGSGAGAGSGAGAGSGAGAGSGAAPGASIKVAVSAGPSAGYGAGAGSGAGAGSGAGAGSGAGAGSGAGAGSGAGAGSGAGAGSGAGAGSGAGAGSGAAPGASIKVAVSAGPSAGYGAGAGSGAGAGSGAGAGSGAGAGSGAGAGSGAGAGSGAGAGSGAGAGSGAGAGSGAAPGASIKVAVSAGPSAGYGAGAGSGAGAGSGAGAGSGAGAGSGAGAGSGAGAGSGAGAGSGAGAGSGAGAGSGAAPGASIKVAVSAGPSAGYGAGAGSGAGAGSGAGAGSGAGAGSGAGAGSGAGAGSGAGAGSGAGAGSGAGAGSGAAPGASIKVAVSAGPSAGYGAGAGSGAGAGSGAGAGSGAGAGSGAGAGSGAGAGSGAGAGSGAGAGSGAGAGSGAAPGASIKVAVSAGPSAGYGAGAGSGAGAGSGAGAMDPGRYQLSAGRYHYQLVWCQK

SEQ ID NO: 33 - protein, 436 aa, Oryctolagus cuniculus
MDPMLTQTPASVSAAVGGTVTIKCQASENIYTSLAWYQQKPGHSPKLLIYSASTLASGVASRFKGSGSGTQFTLTISGVQCDDAATYYCQCSAYGRSGNSFGGGTEVVVNGDPVAPTVLIFPPAADQVATGTVTIVCVANKYFPDVTVTWEVDGTTQTTGIENSKTPQNSADCTYNLSSTLTLTSTQYNSHKEYTCKVTQGTTSVVQSFNRGDCMQSLEESGGRLVTPGTPLTLTCTVSGIDLSRYAMGWVRQAPGKGLEWIAMINGYGTTYYASWAKGRFTISRTSTTVDLKITSPTTEDTATYFCVRYPESSSMFDLWGQGTLVTVSSGQPKAPSVFPLAPCCGDTPSSTVTLGCLVKGYLPEPVTVTWNSGTLTNGVRTFPSVRQSSGLYSLSSVVSVTSSSQPVTCNVAHPATNTKVDKTVAPSTCSKPTCP

SEQ ID NO: 34 - protein, 605 aa, Aspergillus niger
MQTLLVSSLVVSLAAALPHYIRSNGIEASLLTDPKDVSGRTVDYIIAGGGLTGLTTAARLTENPNISVLVIESGSYESDRGPIIEDLNAYGDIFGSSVDHAYETVELATNNQTALIRSGNGLGGSTLVNGGTWTRPHKAQVDSWETVFGNEGWNWDNVAAYSLQAERARAPNAKQIAAGHYFNASCHGVNGTVHAGPRDTGDDYSPIVKALMSAVEDRGVPTKKDFGCGDPHGVSMFPNTLHEDQVRSDAAREWLLPNYQRPNLQVLTGQYVGKVLLSQNGTTPRAVGVEFGTHKGNTHNVYAKHEVLLAAGSAVSPTILEYSGIGMKSILEPLGIDTVVDLPVGLNLQDQTTATVRSRITSAGAGQGQAAWFATFNETFGDYSEKAHELLNTKLEQWAEEAVARGGFHNTTALLIQYENYRDWIVNHNVAYSELFLDTAGVASFDVWDLLPFTRGYVHILDKDPYLHHFAYDPQYFLNELDLLGQAAATQLARNISNSGAMQTYFAGETIPGDNLAYDADLSAWTEYIPYHFRPNYHGVGTCSMMPKEMGGVVDNAARVYGVQGLRVIDGSIPPTQMSSHVMTVFYAMALKISDAILEDYASMQ

SEQ ID NO: 35 - protein, 607 aa, Bos taurus
MKWVTFISLLLLFSSAYSRGVFRRDTHKSEIAHRFKDLGEEHFKGLVLIAFSQYLQQCPFDEHVKLVNELTEFAKTCVADESHAGCEKSLHTLFGDELCKVASLRETYGDMADCCEKQEPERNECFLSHKDDSPDLPKLKPDPNTLCDEFKADEKKFWGKYLYEIARRHPYFYAPELLYYANKYNGVFQECCQAEDKGACLLPKIETMREKVLASSARQRLRCASIQKFGERALKAWSVARLSQKFPKAEFVEVTKLVTDLTKVHKECCHGDLLECADDRADLAKYICDNQDTISSKLKECCDKPLLEKSHCIAEVEKDAIPENLPPLTADFAEDKDVCKNYQEAKDAFLGSFLYEYSRRHPEYAVSVLLRLAKEYEATLEECCAKDDPHACYSTVFDKLKHLVDEPQNLIKQNCDQFEKLGEYGFQNALIVRYTRKVPQVSTPTLVEVSRSLGKVGTRCCTKPESERMPCTEDYLSLILNRLCVLHEKTPVSEKVTKCCTESLVNRRPCFSALTPDETYVPKAFDEKLFTFHADICTLPDTEKQIKKQTALVELLKHKPKATEEQLKTVMENFVAFVDKCCAADDKEACFAVEGPKLVVSTQTALA